European Patent Application EP 4 621 051 A1, published September 24, 2025. Title: Novel acetolactate synthase variant and a method for producing L-glutamic acid using the same. Applicant: CJ CheilJedang Corporation. The sequence listing filed with the application follows.

SEQUENCE LISTING (8 sequences)

SEQ ID NO: 1 - protein, 601 aa, Corynebacterium glutamicum
MTGAQAIVRSLEELNADIVFGIPGGAVLPVYDPLYSSTKVRHVLVRHEQGAGHAATGYAQVTGRVGVCIATSGPGATNLVTPIADANLDSVPMVAITGQVGSSLLGTDAFQEADIRGITMPVTKHNFMVTNPNDIPQALAEAFHLAITGRPGPVLVDIPKDVQNAELDFVWPPKIDLPGYRPVSTPHARQIEQAVKLIGESKKPVLYVGGGVIKADAHEELRAFAEHTGIPVVTTLMALGTFPESHELHMGMPGMHGTVSAVGALQRSDLLIAIGSRFDDRVTGDVDTFAPDAKIIHADIDPAEIGKIKQVEVPIVGDAREVLARLLETTKASKAESEDISEWVDYLKGLKARFPRGYDEQPGDLLAPQFVIETLSKEVGPDAIYCAGVGQHQMWAAQFVDFEKPRTWLNSGGLGTMGYAVPAALGAKAGAPDKEVWAIDGDGCFQMTNQELTTAAVEGFPIKIALINNGNLGMVRQWQTLFYEGRYSNTKLRNQGEYMPDFVTLSEGLGCVAIRVTKAEEVLPAIQKAREINDRPVVIDFIVGEDAQVWPMVSAGSSNSDIQYALGLRPFFDGDESAAEDPADIHEAVSDIDAAVESTEA

SEQ ID NO: 2 - DNA, 1806 bp, Corynebacterium glutamicum
  source 1..1806: mol_type = genomic DNA
atgacaggtgcacaggcaattgttcgatcgctcgaggagcttaacgccgacatcgtgttcggtattcctggtggtgcggtgctaccggtgtatgacccgctctattcctccacaaaggtgcgccacgtcctagtgcgccacgagcagggcgcaggccacgcagcaaccggctacgcgcaggttactggacgcgttggcgtctgcattgcaacctctggcccaggcgcaaccaacttggttaccccaatcgctgatgcaaacttggactccgttcccatggttgccatcaccggccaggtcggaagtagcctgctgggtaccgatgctttccaggaagccgatatccgcggcatcaccatgccagtgaccaagcacaacttcatggtcaccaaccccaacgacattccacaggcattggctgaggcattccacctcgcgattactggtcgccctggtcctgttctagtggatatccccaaggatgttcagaacgctgaattggatttcgtctggccaccaaagatcgacctgccaggctaccgcccagtttcaacaccgcatgctcgacagattgagcaggctgtcaaactgatcggtgagtctaagaagcctgtcctttacgttggcggcggcgttatcaaggctgatgcccacgaagagcttcgtgcgttcgctgagcacaccggcattccagttgtcaccacattgatggcgctgggaaccttcccagagtcccacgagctgcacatgggtatgccaggcatgcatggcactgtgtccgctgttggtgcactgcagcgcagcgacctgctgattgctatcggctcccgctttgatgaccgcgtcaccggtgacgttgacactttcgcacctgatgccaagatcattcacgccgacattgatcctgccgaaatcggcaagatcaagcaggttgaggttccaatcgtgggcgatgcccgcgaggttcttgctcgtctgctcgaaaccaccaaggcaagcaaggcagagtctgaggacatctccgagtgggttgactacctcaagggcctcaaggcacgtttcccacgtggctacgacgagcagccaggcgatctgctggcaccacagtttgtcattgaaaccctgtccaaggaagttggccccgacgcaatttactgcgccggcgttggccagcaccagatgtgggcagctcagttcgttgacttcgaaaagccacgcacctggctcaactccggtggactgggcaccatgggctacgcagttcctgcggctcttggagcaaaggctggcgcacctgacaaggaagtctgggctatcgacggcgacggctgtttccagatgaccaaccaggaactcaccaccgccgcagttgaaggtttccccattaagatcgcactaatcaacaacggaaacctgggtatggttcgccaatggcagaccctattctatgaaggacggtactcaaatactaaacttcgtaaccagggcgagtacatgcccgactttgttaccctttctgagggacttggctgtgttgccatccgcgtcaccaaagcggaggaagtactgccagccatccaaaaggctcgagagatcaacgaccgcccagtagtcatcgacttcatcgtcggtgaagacgcacaggtatggccaatggtgtctgctggatcatccaactccgatatccagtacgcactcggattgcgcccattctttgatggtgatgaatctgcagcagaagatcctgccgacattcacgaagccgtcagcgacattgatgccgccgttgaatcgaccgaggcataa

SEQ ID NO: 3 - protein, 601 aa, synthetic construct
MTGAQAIVRSLEELNADIVFGIPGGAVLPVYDPLYSSTKVRHVLVRHEQGAGHAATGYAQVTGRVGVCIATSGPGATNLVTPIADANLDSVPMVAITGQVGSSLLGTDAFQEADIRGITMPVTKHNFMVTNPNDIPQALAEAFHLAITGRPGPVLVDIPKDVQNAELDFVWPPKIDLPGYRPVSTPHARQIEQAVKLIGESKKPVLYVGGGVIKADAHEELRAFAEHTGIPVVTTLMALGTFPESHELHMGMPGMHGTVSAVGALQRSDLLIAIGSRFDDRVTGDVDTFAPDAKIIHVDIDPAEIGKIKQVEVPIVGDAREVLARLLETTKASKAESEDISEWVDYLKGLKARFPRGYDEQPGDLLAPQFVIETLSKEVGPDAIYCAGVGQHQMWAAQFVDFEKPRTWLNSGGLGTMGYAVPAALGAKAGAPDKEVWAIDGDGCFQMTNQELTTAAVEGFPIKIALINNGNLGMVRQWQTLFYEGRYSNTKLRNQGEYMPDFVTLSEGLGCVAIRVTKAEEVLPAIQKAREINDRPVVIDFIVGEDAQVWPMVSAGSSNSDIQYALGLRPFFDGDESAAEDPADIHEAVSDIDAAVESTEA

SEQ ID NO: 4 - DNA, 1806 bp, synthetic construct
  source 1..1806: mol_type = other DNA
atgacaggtgcacaggcaattgttcgatcgctcgaggagcttaacgccgacatcgtgttcggtattcctggtggtgcggtgctaccggtgtatgacccgctctattcctccacaaaggtgcgccacgtcctagtgcgccacgagcagggcgcaggccacgcagcaaccggctacgcgcaggttactggacgcgttggcgtctgcattgcaacctctggcccaggcgcaaccaacttggttaccccaatcgctgatgcaaacttggactccgttcccatggttgccatcaccggccaggtcggaagtagcctgctgggtaccgatgctttccaggaagccgatatccgcggcatcaccatgccagtgaccaagcacaacttcatggtcaccaaccccaacgacattccacaggcattggctgaggcattccacctcgcgattactggtcgccctggtcctgttctagtggatatccccaaggatgttcagaacgctgaattggatttcgtctggccaccaaagatcgacctgccaggctaccgcccagtttcaacaccgcatgctcgacagattgagcaggctgtcaaactgatcggtgagtctaagaagcctgtcctttacgttggcggcggcgttatcaaggctgatgcccacgaagagcttcgtgcgttcgctgagcacaccggcattccagttgtcaccacattgatggcgctgggaaccttcccagagtcccacgagctgcacatgggtatgccaggcatgcatggcactgtgtccgctgttggtgcactgcagcgcagcgacctgctgattgctatcggctcccgctttgatgaccgcgtcaccggtgacgttgacactttcgcacctgatgccaagatcattcacgtcgacattgatcctgccgaaatcggcaagatcaagcaggttgaggttccaatcgtgggcgatgcccgcgaggttcttgctcgtctgctcgaaaccaccaaggcaagcaaggcagagtctgaggacatctccgagtgggttgactacctcaagggcctcaaggcacgtttcccacgtggctacgacgagcagccaggcgatctgctggcaccacagtttgtcattgaaaccctgtccaaggaagttggccccgacgcaatttactgcgccggcgttggccagcaccagatgtgggcagctcagttcgttgacttcgaaaagccacgcacctggctcaactccggtggactgggcaccatgggctacgcagttcctgcggctcttggagcaaaggctggcgcacctgacaaggaagtctgggctatcgacggcgacggctgtttccagatgaccaaccaggaactcaccaccgccgcagttgaaggtttccccattaagatcgcactaatcaacaacggaaacctgggtatggttcgccaatggcagaccctattctatgaaggacggtactcaaatactaaacttcgtaaccagggcgagtacatgcccgactttgttaccctttctgagggacttggctgtgttgccatccgcgtcaccaaagcggaggaagtactgccagccatccaaaaggctcgagagatcaacgaccgcccagtagtcatcgacttcatcgtcggtgaagacgcacaggtatggccaatggtgtctgctggatcatccaactccgatatccagtacgcactcggattgcgcccattctttgatggtgatgaatctgcagcagaagatcctgccgacattcacgaagccgtcagcgacattgatgccgccgttgaatcgaccgaggcataa

SEQ ID NO: 5 - DNA, 32 bp, synthetic construct
  source 1..32: mol_type = other DNA
cggtacccggggatccaggcattggctgaggc

SEQ ID NO: 6 - DNA, 36 bp, synthetic construct
  source 1..36: mol_type = other DNA
ggcaggatcaatgtcgacgtgaatgatcttggcatc

SEQ ID NO: 7 - DNA, 35 bp, synthetic construct
  source 1..35: mol_type = other DNA
tcgacattgatcctgccgaaatcggcaagatcaag

SEQ ID NO: 8 - DNA, 33 bp, synthetic construct
  source 1..33: mol_type = other DNA
atgcctgcaggtcgacgatcttaatggggaaac